European Patent Application EP 4 306 535 A1, published January 17, 2024. Title: Compounds and salts thereof and antibody obtained by the same. Applicant: Ajinomoto Co., Inc. The sequence listing filed with the application follows.

SEQUENCE LISTING (6 sequences)

SEQ ID NO: 1 - protein, 17 aa, Artificial Sequence
  Peptide having an affinity to Fc region of human IgG.  The amino acid residue at N-terminus may be acetylated, the amino acid residue at C-terminus may be aminated and two cysteine residues may be linked by disulfide bridge.
  MISC_FEATURE (1)..(1): absent, or any amino acid other than lysine and cysteine
  MISC_FEATURE (2)..(2): absent, or any amino acid other than lysine and cysteine
  MISC_FEATURE (3)..(3): absent, or any amino acid other than lysine and cysteine
  MISC_FEATURE (5)..(5): alanine, glycine, leucine, proline, arginine, valine, asparagine, glutamic acid, or phenylalanine
  MISC_FEATURE (6)..(6): tyrosine, tryptophan, histidine, or phenylalanine
  MISC_FEATURE (7)..(7): histidine, phenylalanine, tyrosine, tryptophan, arginine, or glycine
  MISC_FEATURE (8)..(8): lysine
  MISC_FEATURE (9)..(9): glycine, serine, asparagine, glutamine, aspartic acid, glutamic acid, phenylalanine, tyrosine, tryptophan, histidine, threonine, leucine, alanine, valine, isoleucine, or arginine
  MISC_FEATURE (10)..(10): glutamine, glutamic acid, asparagine, aspartic acid, proline, glycine, arginine, phenylalanine, or histidine
  MISC_FEATURE (15)..(15): absent, or any amino acid other than lysine and cysteine
  MISC_FEATURE (16)..(16): absent, or any amino acid other than lysine and cysteine
  MISC_FEATURE (17)..(17): absent, or any amino acid other than lysine and cysteine
XXXCXXXXXXIIWCXXX

SEQ ID NO: 2 - protein, 17 aa, Artificial Sequence
  Affinity peptide
RGNCAYHKGQIIWCTYH

SEQ ID NO: 3 - protein, 15 aa, Artificial Sequence
  Affinity peptide
PNLNEEQRNARIRSI

SEQ ID NO: 4 - protein, 34 aa, Artificial Sequence
  Affinity peptide
FNMQCQRRFYEALHDPNLNEEQRNARIRSIKDDC

SEQ ID NO: 5 - protein, 34 aa, Artificial Sequence
  Affinity peptide
FNMQCQRRFYEALHDPNLNEEQRNARIRSIKEEC

SEQ ID NO: 6 - protein, 32 aa, Artificial Sequence
  Affinity peptide
  misc_feature (29)..(29): Xaa can be any naturally occurring amino acid
  MISC_FEATURE (32)..(32): Ornithine
MQCQRRFYEALHDPNLNEEQRNARIRSIXEEC